European Patent Application EP 4 613 781 A1, published September 10, 2025. Title: IMMUNE REJECTION-RESISTANT ENGINEERED CELL. Applicant: NANJING BIOHENG BIOTECH CO., LTD. Application EP. The sequence listing filed with the application follows.

SEQUENCE LISTING (69 sequences)

SEQ ID NO: 1 - protein, 7 aa, synthetic construct
  source 1..7: note = Anti-FasL-1 CDR1-H
GYIFIRH

SEQ ID NO: 2 - protein, 6 aa, synthetic construct
  source 1..6: note = Anti-FasL-1 CDR2-H
NAYNGN

SEQ ID NO: 3 - protein, 11 aa, synthetic construct
  source 1..11: note = Anti-FasL-1 CDR3-H
ETMVRGVPLDY

SEQ ID NO: 4 - protein, 12 aa, synthetic construct
  source 1..12: note = Anti-FasL-1 CDR1-L
RASQSVSSSYLA

SEQ ID NO: 5 - protein, 7 aa, synthetic construct
  source 1..7: note = Anti-FasL-1 CDR2-L
GASSRAT

SEQ ID NO: 6 - protein, 9 aa, synthetic construct
  source 1..9: note = Anti-FasL-1 CDR3-L
QQYGSSPWT

SEQ ID NO: 7 - protein, 120 aa, synthetic construct
  source 1..120: note = Anti-FasL-1 VH
QVQLVQSGAEVKKPGASVKVSCKASGYIFIRHGITWVRQAPGQGLEWMGWINAYNGNTNYAQKVQGRVTMTTDKSTSTAYMELRSLRSDDAAVYYCARETMVRGVPLDYWGQGTLVTVSS

SEQ ID NO: 8 - protein, 109 aa, synthetic construct
  source 1..109: note = Anti-FasL-1 VL
EIVLTQSPGTLSLSPGERATLSCRASQSVSSSYLAWYQQKPGQAPRLLIYGASSRATGIPDRFSGSGSGTDFTLTISRLEPEDFAVYYCQQYGSSPWTFGQGTKVEIKR

SEQ ID NO: 9 - protein, 244 aa, synthetic construct
  source 1..244: note = Anti-FasL-1 scFv
QVQLVQSGAEVKKPGASVKVSCKASGYIFIRHGITWVRQAPGQGLEWMGWINAYNGNTNYAQKVQGRVTMTTDKSTSTAYMELRSLRSDDAAVYYCARETMVRGVPLDYWGQGTLVTVSSGGGGSGGGGSGGGGSEIVLTQSPGTLSLSPGERATLSCRASQSVSSSYLAWYQQKPGQAPRLLIYGASSRATGIPDRFSGSGSGTDFTLTISRLEPEDFAVYYCQQYGSSPWTFGQGTKVEIKR

SEQ ID NO: 10 - protein, 7 aa, synthetic construct
  source 1..7: note = Anti-FasL-2 CDR1-H
GYIFISH

SEQ ID NO: 11 - protein, 6 aa, synthetic construct
  source 1..6: note = Anti-FasL-2 CDR1-H
NAYSGN

SEQ ID NO: 12 - protein, 11 aa, synthetic construct
  source 1..11: note = Anti-FasL-2 CDR3-H
ETMVRGVPCDY

SEQ ID NO: 13 - protein, 120 aa, synthetic construct
QVQLVQSGAEVKKPGASVKVSCKASGYIFISHGISWVRQAPGQGLEWMGWINAYSGNTNYAQKLQGRVTMTTDRSTSTAYMELRSLRSDDTAVYYCARETMVRGVPCDYWGQGTLVTVSS

SEQ ID NO: 14 - protein, 244 aa, synthetic construct
QVQLVQSGAEVKKPGASVKVSCKASGYIFISHGISWVRQAPGQGLEWMGWINAYSGNTNYAQKLQGRVTMTTDRSTSTAYMELRSLRSDDTAVYYCARETMVRGVPCDYWGQGTLVTVSSGGGGSGGGGSGGGGSEIVLTQSPGTLSLSPGERATLSCRASQSVSSSYLAWYQQKPGQAPRLLIYGASSRATGIPDRFSGSGSGTDFTLTISRLEPEDFAVYYCQQYGSSPWTFGQGTKVEIKR

SEQ ID NO: 15 - protein, 27 aa, synthetic construct
  source 1..27: note = CD28 transmembrane domain
FWVLVVVGGVLACYSLLVTVAFIIFWV

SEQ ID NO: 16 - protein, 25 aa, synthetic construct
  source 1..25: note = CD8a transmembrane domain
IYIWAPLAGTCGVLLLSLVITLYCK

SEQ ID NO: 17 - protein, 21 aa, synthetic construct
  source 1..21: note = mCD8a transmembrane domain
IWAPLAGICVALLLSLIITLI

SEQ ID NO: 18 - protein, 41 aa, synthetic construct
  source 1..41: note = CD28 costimulatory domain
RSKRSRLLHSDYMNMTPRRPGPTRKHYQPYAPPRDFAAYRS

SEQ ID NO: 19 - protein, 40 aa, synthetic construct
  source 1..40: note = 4-1BB costimulatory domain
RGRKKLLYIFKQPFMRPVQTTQEEDGCSCRFPEEEEGGCE

SEQ ID NO: 20 - protein, 42 aa, synthetic construct
  source 1..42: note = m4-1BB costimulatory domain
RKKFPHIFKQPFKKTTGAAQEEDACSCRCPQEEEGGGGGYEL

SEQ ID NO: 21 - protein, 114 aa, synthetic construct
  source 1..114: note = CD3zm intracellular region
LRVKFSRSADAPAYQQGQNQLFNELNLGRREEFDVLDKRRGRDPEMGGKPQRRKNPQEGLYNELQKDKMAEAYSEIGMKGERRRGKGHDGLFQGLSTATKDTFDALHMQALPPR

SEQ ID NO: 22 - protein, 113 aa, synthetic construct
  source 1..113: note = CD3z intracellular region
LRVKFSRSADAPAYQQGQNQLYNELNLGRREEYDVLDKRRGRDPEMGGKPRRKNPQEGLYNELQKDKMAEAYSEIGMKGERRRGKGHDGLYQGLSTATKDTYDALHMQALPPR

SEQ ID NO: 23 - protein, 109 aa, synthetic construct
  source 1..109: note = mCD3z intracellular region
SRSAETAANLQDPNQLYNELNLGRREEYDVLEKKRARDPEMGGKQQRRRNPQEGVYNALQKDKMAEAYSEIGTKGERRRGKGHDGLYQGLSTATKDTYDALHMQTLAPR

SEQ ID NO: 24 - protein, 20 aa, synthetic construct
  source 1..20: note = B2M signal peptide
MSRSVALAVLALLSLSGLEA

SEQ ID NO: 25 - protein, 21 aa, synthetic construct
  source 1..21: note = CD8a signal peptide
MALPVTALLLPLALLLHAARP

SEQ ID NO: 26 - protein, 24 aa, synthetic construct
  source 1..24: note = mCD8a signal peptide
MASPLTRFLSLNLLLLGESIILGS

SEQ ID NO: 27 - protein, 39 aa, synthetic construct
  source 1..39: note = CD28 hinge region
IEVMYPPPYLDNEKSNGTIIHVKGKHLCPSPLFPGPSKP

SEQ ID NO: 28 - protein, 45 aa, synthetic construct
  source 1..45: note = CD8a hinge region
TTTPAPRPPTPAPTIASQPLSLRPEACRPAAGGAVHTRGLDFACD

SEQ ID NO: 29 - protein, 45 aa, synthetic construct
  source 1..45: note = mCD8a hinge region
TTTKPVLRTPSPVHPTGTSQPQRPEDCRPRGSVKGTGLDFACDIY

SEQ ID NO: 30 - protein, 12 aa, synthetic construct
  source 1..12: note = IgG4 hinge region
ESKYGPPCPPCP

SEQ ID NO: 31 - protein, 18 aa, synthetic construct
  source 1..18: note = T2A
EGRGSLLTCGDVEENPGP

SEQ ID NO: 32 - protein, 7 aa, synthetic construct
  source 1..7: note = CD19 CDR-H1
GVSLPDY

SEQ ID NO: 33 - protein, 5 aa, synthetic construct
  source 1..5: note = CD19 CDR-H2
WGSET

SEQ ID NO: 34 - protein, 12 aa, synthetic construct
  source 1..12: note = CD19 CDR-H3
HYYYGGSYAMDY

SEQ ID NO: 35 - protein, 11 aa, synthetic construct
  source 1..11: note = CD19 CDR-L1
RASQDISKYLN

SEQ ID NO: 36 - protein, 7 aa, synthetic construct
  source 1..7: note = CD19 CDR-L2
HTSRLHS

SEQ ID NO: 37 - protein, 9 aa, synthetic construct
  source 1..9: note = CD19 CDR-L3
QQGNTLPYT

SEQ ID NO: 38 - protein, 120 aa, synthetic construct
  source 1..120: note = CD19 VH
EVKLQESGPGLVAPSQSLSVTCTVSGVSLPDYGVSWIRQPPRKGLEWLGVIWGSETTYYNSALKSRLTIIKDNSKSQVFLKMNSLQTDDTAIYYCAKHYYYGGSYAMDYWGQGTSVTVSS

SEQ ID NO: 39 - protein, 107 aa, synthetic construct
  source 1..107: note = CD19 VL
DIQMTQTTSSLSASLGDRVTISCRASQDISKYLNWYQQKPDGTVKLLIYHTSRLHSGVPSRFSGSGSGTDYSLTISNLEQEDIATYFCQQGNTLPYTFGGGTKLEIT

SEQ ID NO: 40 - protein, 120 aa, synthetic construct
  source 1..120: note = hCD19 VH-1
QVTLKESGPVLVKPTETLTLTCTVSGVSLPDYGVSWIRQPPGKALEWLAVIWGSETTYYNSALKSRLTISKDTSKSQVVLTMTNMDPVDTATYYCARHYYYGGSYAMDYWGQGTMVTVSS

SEQ ID NO: 41 - protein, 106 aa, synthetic construct
  source 1..106: note = hCD19 VL-1
DIQMTQSPSSLSASVGDRVTITCRASQDISKYLNWYQQKPGKAPKLLLYHTSRLHSGVPSRFSGSGSGTDYTLTISSLQQEDFATYYCQQGNTLPYTFGQGTKVEI

SEQ ID NO: 42 - protein, 120 aa, synthetic construct
  source 1..120: note = hCD19 VH-2
QVTLKESGPVLVKPTETLTLTCTVSGVSLPDYGVSWIRQPPGKALEWLAVIWGSETTYYNSALKSRLTISKDTSKSQVVLTMTNMDPVDTATYYCAKHYYYGGSYAMDYWGQGTMVTVSS

SEQ ID NO: 43 - protein, 106 aa, synthetic construct
  source 1..106: note = hCD19 VL-2
DIQMTQSPSSVSASVGDRVTITCRASQDISKYLNWYQQKPGKAPKLLIYHTSRLHSGVPSRFSGSGSGTDFTLTISSLQPEDFATYYCQQGNTLPYTFGQGTRLEI

SEQ ID NO: 44 - protein, 242 aa, synthetic construct
  source 1..242: note = CD19 scfv
DIQMTQTTSSLSASLGDRVTISCRASQDISKYLNWYQQKPDGTVKLLIYHTSRLHSGVPSRFSGSGSGTDYSLTISNLEQEDIATYFCQQGNTLPYTFGGGTKLEITGGGGSGGGGSGGGGSEVKLQESGPGLVAPSQSLSVTCTVSGVSLPDYGVSWIRQPPRKGLEWLGVIWGSETTYYNSALKSRLTIIKDNSKSQVFLKMNSLQTDDTAIYYCAKHYYYGGSYAMDYWGQGTSVTVSS

SEQ ID NO: 45 - protein, 241 aa, synthetic construct
  source 1..241: note = hCD19-1 VH1-VL1
QVTLKESGPVLVKPTETLTLTCTVSGVSLPDYGVSWIRQPPGKALEWLAVIWGSETTYYNSALKSRLTISKDTSKSQVVLTMTNMDPVDTATYYCARHYYYGGSYAMDYWGQGTMVTVSSGGGGSGGGGSGGGGSDIQMTQSPSSLSASVGDRVTITCRASQDISKYLNWYQQKPGKAPKLLLYHTSRLHSGVPSRFSGSGSGTDYTLTISSLQQEDFATYYCQQGNTLPYTFGQGTKVEI

SEQ ID NO: 46 - protein, 240 aa, synthetic construct
  source 1..240: note = hCD19-2 VL1-VH1
DIQMTQSPSSLSASVGDRVTITCRASQDISKYLNWYQQKPGKAPKLLLYHTSRLHSGVPRFSGSGSGTDYTLTISSLQQEDFATYYCQQGNTLPYTFGQGTKVEIGGGGSGGGGSGGGGSQVTLKESGPVLVKPTETLTLTCTVSGVSLPDYGVSWIRQPPGKALEWLAVIWGSETTYYNSALKSRLTISKDTSKSQVVLTMTNMDPVDTATYYCARHYYYGGSYAMDYWGQGTMVTVSS

SEQ ID NO: 47 - protein, 241 aa, synthetic construct
  source 1..241: note = hCD19-3 VH1-VL1
QVTLKESGPVLVKPTETLTLTCTVSGVSLPDYGVSWIRQPPGKALEWLAVIWGSETTYYNSALKSRLTISKDTSKSQVVLTMTNMDPVDTATYYCAKHYYYGGSYAMDYWGQGTMVTVSSGGGGSGGGGSGGGGSDIQMTQSPSSVSASVGDRVTITCRASQDISKYLNWYQQKPGKAPKLLIYHTSRLHSGVPSRFSGSGSGTDFTLTISSLQPEDFATYYCQQGNTLPYTFGQGTRLEI

SEQ ID NO: 48 - protein, 241 aa, synthetic construct
  source 1..241: note = hCD19-4 VL1-VH1
DIQMTQSPSSVSASVGDRVTITCRASQDISKYLNWYQQKPGKAPKLLIYHTSRLHSGVPSRFSGSGSGTDFTLTISSLQPEDFATYYCQQGNTLPYTFGQGTRLEIGGGGSGGGGSGGGGSQVTLKESGPVLVKPTETLTLTCTVSGVSLPDYGVSWIRQPPGKALEWLAVIWGSETTYYNSALKSRLTISKDTSKSQVVLTMTNMDPVDTATYYCAKHYYYGGSYAMDYWGQGTMVTVSS

SEQ ID NO: 49 - protein, 190 aa, synthetic construct
  source 1..190: note = Fas
MLGIWTLLPLVLTSVARLSSKSVNAQVTDINSKGLELRKTVTTVETQNLEGLHHDGQFCHKPCPPGERKARDCTVNGDEPDCVPCQEGKEYTDKAHFSSKCRRCRLCDEGHGLEVEINCTRTQNTKCRCKPNFFCNSTVCEHCDPCTKCEHGIIKECTLTSNTKCKEEGSRSNLGWLCLLLLPIPLIVWV

SEQ ID NO: 50 - protein, 7 aa, synthetic construct
  source 1..7: note = SIRPa CDR1-H
GFNISYY

SEQ ID NO: 51 - protein, 6 aa, synthetic construct
  source 1..6: note = SIRPa CDR2-H
YSSFGY

SEQ ID NO: 52 - protein, 20 aa, synthetic construct
  source 1..20: note = SIRPa CDR3-H
FTFPGLFTGFFGAYLGSLDY

SEQ ID NO: 53 - protein, 11 aa, synthetic construct
  source 1..11: note = SIRPa CDR1-L
RASQSVSSAVA

SEQ ID NO: 54 - protein, 7 aa, synthetic construct
  source 1..7: note = SIRPa CDR2-L
SASSLYS

SEQ ID NO: 55 - protein, 12 aa, synthetic construct
  source 1..12: note = SIRPa CDR3-L
QQAVNWVGALVT

SEQ ID NO: 56 - protein, 129 aa, synthetic construct
  source 1..129: note = SIRPa VH
EVQLVESGGGLVQPGGSLRLSCAASGFNISYYFIHWVRQAPGKGLEWVASVYSSFGYTYYADSVKGRFTISADTSKNTAYLQMNSLRAEDTAVYYCARFTFPGLFTGFFGAYLGSLDYWGQGTLVTVSS

SEQ ID NO: 57 - protein, 111 aa, synthetic construct
  source 1..111: note = SIRPa VL
DIQMTQSPSSLSASVGDRVTITCRASQSVSSAVAWYQQKPGKAPKLLIYSASSLYSGVPSRFSGSRSGTDFTLTISSLQPEDFATYYCQQAVNWVGALVTFGQGTKVEIKR

SEQ ID NO: 58 - protein, 252 aa, synthetic construct
  source 1..252: note = SIRPa scFv
EVQLVESGGGLVQPGGSLRLSCAASGFNISYYFIHWVRQAPGKGLEWVASVYSSFGYTYYADSVKGRFTISADTSKNTAYLQMNSLRAEDTAVYYCARFTFPGLFTGFFGAYLGSLDYWGQGTLVTVSSGGGSGGGSGGGSDIQMTQSPSSLSASVGDRVTITCRASQSVSSAVAWYQQKPGKAPKLLIYSASSLYSGVPSRFSGSRSGTDFTLTISSLQPEDFATYYCQQAVNWVGALVTFGQGTKVEIKR

SEQ ID NO: 59 - protein, 7 aa, synthetic construct
  source 1..7: note = IRP60 CDR1-H
GYTFTSY

SEQ ID NO: 60 - protein, 6 aa, synthetic construct
  source 1..6: note = IRP60 CDR2-H
DPSDSY

SEQ ID NO: 61 - protein, 15 aa, synthetic construct
  source 1..15: note = IRP60 CDR3-H
WGMAYGTSSYWYFDV

SEQ ID NO: 62 - protein, 11 aa, synthetic construct
  source 1..11: note = IRP60 CDR1-L
RASQDISNYLN

SEQ ID NO: 63 - protein, 7 aa, synthetic construct
  source 1..7: note = IRP60 CDR2-L
YTSRLHS

SEQ ID NO: 64 - protein, 9 aa, synthetic construct
  source 1..9: note = IRP60 CDR3-L
QQGNTLPWT

SEQ ID NO: 65 - protein, 125 aa, synthetic construct
  source 1..125: note = IRP60 VH
EVQLQQSGAELVKPGASVKLSCKASGYTFTSYWMQWVKQRPGQGLEWIGEIDPSDSYTNYNQKFKGKATLTVDTSSSTTYMQLSSLTSEDSAVYYCARWGMAYGTSSYWYFDVWGTGTTVTVSSA

SEQ ID NO: 66 - protein, 107 aa, synthetic construct
  source 1..107: note = IRP60 VL
DIQMTQTTSSLSASLGDRVTISCRASQDISNYLNWYQQKPDGTVKLLIYYTSRLHSGVPSRFSGSGSGTDYSLTISNLEQEDIATYFCQQGNTLPWTFGGGTKLEIK

SEQ ID NO: 67 - protein, 244 aa, synthetic construct
  source 1..244: note = IRP60 scFv
EVQLQQSGAELVKPGASVKLSCKASGYTFTSYWMQWVKQRPGQGLEWIGEIDPSDSYTNYNQKFKGKATLTVDTSSSTTYMQLSSLTSEDSAVYYCARWGMAYGTSSYWYFDVWGTGTTVTVSSAGGGSGGGSGGGSDIQMTQTTSSLSASLGDRVTISCRASQDISNYLNWYQQKPDGTVKLLIYYTSRLHSGVPSRFSGSGSGTDYSLTISNLEQEDIATYFCQQGNTLPWTFGGGTKLEIK

SEQ ID NO: 68 - protein, 289 aa, synthetic construct
  source 1..289: note = CD47
MWPLVAALLLGSACCGSAQLLFNKTKSVEFTFCNDTVVIPCFVTNMEAQNTTEVYVKWKFKGRDIYTFDGALNKSTVPTDFSSAKIEVSQLLKGDASLKMDKSDAVSHTGNYTCEVTELTREGETIIELKYRVVSWFSPNENILIVIFPIFAILLFWGQFGIKTLKYRSGGMDEKTIALLVAGLVITVIVIVGAILFVPGEYSLKNATGLGLIVTSTGILILLHYYVFSTAIGLTSFVIAILVIQVIAYILAVVGLSLCIAACIPMHGPLLISGLSILALAQLLGLVYM

SEQ ID NO: 69 - protein, 142 aa, synthetic construct
  source 1..142: note = CD47
MWPLVAALLLGSACCGSAQLLFNKTKSVEFTFCNDTVVIPCFVTNMEAQNTTEVYVKWKFKGRDIYTFDGALNKSTVPTDFSSAKIEVSQLLKGDASLKMDKSDAVSHTGNYTCEVTELTREGETIIELKYRVVSWFSPNEN